European Patent Specification EP 3 006 042 B1, published May 8, 2024. Title: A composition for treating inflammatory diseases comprising an anti-myosin regulatory light chain polypeptide antibody. Applicant: NATIONAL UNIVERSITY CORPORATION CHIBA UNIVERSITY. The sequence listing filed with the application follows.

SEQUENCE LISTING (24 sequences)

SEQ ID NO: 1 - DNA, 519 bp, homo sapiens
  misc_feature: nucleotide sequence of DNA encoding human myl9 isoform a
  CDS (1)..(519)
atgtccagcaagcgggccaaagccaagaccaccaagaagcggccacagcgggccacatccaatgtcttcgcaatgtttgaccagtcccagatccaggagtttaaggaggctttcaacatgattgaccagaaccgtgatggcttcattgacaaggaggacctgcacgacatgctggcctcgctggggaagaaccccacagacgaatacctggagggcatgatgagcgaggccccggggcccatcaacttcaccatgttcctcaccatgtttggggagaagctgaacggcacggaccccgaggatgtgattcgcaacgcctttgcctgcttcgacgaggaagcctcaggtttcatccatgaggaccacctccgggagctgctcaccaccatgggtgaccgcttcacagatgaggaagtggacgagatgtaccgggaggcacccattgataagaaaggcaacttcaactacgtggagttcacccgcatcctcaaacatggcgccaaggataaagacgactag

SEQ ID NO: 2 - protein, 172 aa, homo sapiens
MSSKRAKAKTTKKRPQRATSNVFAMFDQSQIQEFKEAFNMIDQNRDGFIDKEDLHDMLASLGKNPTDEYLEGMMSEAPGPINFTMFLTMFGEKLNGTDPEDVIRNAFACFDEEASGFIHEDHLRELLTTMGDRFTDEEVDEMYREAPIDKKGNFNYVEFTRILKHGAKDKDD

SEQ ID NO: 3 - DNA, 357 bp, homo sapiens
  misc_feature: nucleotide sequence of DNA encoding human myl9 isoform b
  CDS (1)..(357)
atgtccagcaagcgggccaaagccaagaccaccaagaagcggccacagcgggccacatccaatgtcttcgcaatgtttgaccagtcccagatccaggagtttaaggaggctttcaacatgattgaccagaaccgtgatggcttcattgacaaggaggacctgcacgacatgctggcctcgctgggtttcatccatgaggaccacctccgggagctgctcaccaccatgggtgaccgcttcacagatgaggaagtggacgagatgtaccgggaggcacccattgataagaaaggcaacttcaactacgtggagttcacccgcatcctcaaacatggcgccaaggataaagacgactag

SEQ ID NO: 4 - protein, 118 aa, homo sapiens
MSSKRAKAKTTKKRPQRATSNVFAMFDQSQIQEFKEAFNMIDQNRDGFIDKEDLHDMLASLGFIHEDHLRELLTTMGDRFTDEEVDEMYREAPIDKKGNFNYVEFTRILKHGAKDKDD

SEQ ID NO: 5 - DNA, 516 bp, homo sapiens
  misc_feature: nucleotide sequence of DNA encoding human myl12 isoform a
  CDS (1)..(516)
atgtcgagcaaaagaacaaagaccaagaccaagaagcgccctcagcgtgcaacatccaatgtgtttgctatgtttgaccagtcgcagattcaggagttcaaagaggccttcaacatgattgatcagaacagagatggtttcatcgacaaggaagatttgcatgatatgcttgcttcattggggaagaatccaactgatgagtatctagatgccatgatgaatgaggctccaggccccatcaatttcaccatgttcctcaccatgtttggtgagaagttaaatggcacagatcctgaagatgtcatcagaaatgcctttgcttgctttgatgaagaagcaactggcaccatacaggaagattacttgagagagctgctgacaaccatgggggatcggtttacagatgaggaagtggatgagctgtacagagaagcacctattgataaaaaggggaatttcaattacatcgagttcacacgcatcctgaaacatggagccaaagacaaagatgactga

SEQ ID NO: 6 - protein, 171 aa, homo sapiens
MSSKRTKTKTKKRPQRATSNVFAMFDQSQIQEFKEAFNMIDQNRDGFIDKEDLHDMLASLGKNPTDEYLDAMMNEAPGPINFTMFLTMFGEKLNGTDPEDVIRNAFACFDEEATGTIQEDYLRELLTTMGDRFTDEEVDELYREAPIDKKGNFNYIEFTRILKHGAKDKDD

SEQ ID NO: 7 - DNA, 519 bp, homo sapiens
  misc_feature: nucleotide sequence of transcript variant 1 encoding human myl12 isoform b
  CDS (1)..(519)
atgtcgagcaaaaaggcaaagaccaagaccaccaagaagcgccctcagcgtgcaacatccaatgtgtttgccatgtttgaccagtcacagattcaggagttcaaagaggccttcaacatgattgatcagaacagagatggcttcatcgacaaggaagatttgcatgatatgcttgcttctctagggaagaatcccactgatgcataccttgatgccatgatgaatgaggccccagggcccatcaatttcaccatgttcctgaccatgtttggtgagaagttaaatggcacagatcctgaagatgtcatcagaaacgcctttgcttgctttgatgaagaagcaacaggcaccattcaggaagattacctaagagagctgctgacaaccatgggggatcggtttacagatgaggaagtggatgagctgtacagagaagcacctattgacaaaaaggggaatttcaattacatcgagttcacacgcatcctgaaacatggagccaaagacaaagatgactga

SEQ ID NO: 8 - protein, 172 aa, homo sapiens
MSSKKAKTKTTKKRPQRATSNVFAMFDQSQIQEFKEAFNMIDQNRDGFIDKEDLHDMLASLGKNPTDAYLDAMMNEAPGPINFTMFLTMFGEKLNGTDPEDVIRNAFACFDEEATGTIQEDYLRELLTTMGDRFTDEEVDELYREAPIDKKGNFNYIEFTRILKHGAKDKDD

SEQ ID NO: 9 - DNA, 519 bp, homo sapiens; identical to SEQ ID NO: 7
  misc_feature: nucleotide sequence of transcript variant 2 encoding human myl12 isoform b
  CDS (1)..(519)

SEQ ID NO: 10 - protein, 172 aa, homo sapiens; identical to SEQ ID NO: 8

SEQ ID NO: 11 - DNA, 519 bp, homo sapiens; identical to SEQ ID NO: 7
  misc_feature: nucleotide sequence of transcript variant 3 encoding human myl12 isoform b
  CDS (1)..(519)

SEQ ID NO: 12 - protein, 172 aa, homo sapiens; identical to SEQ ID NO: 8

SEQ ID NO: 13 - DNA, 519 bp, mus musculus
  misc_feature: nucleotide sequence of DNA encoding mouse myl9
  CDS (1)..(519)
atgtcgagcaagagagccaaggccaagaccaccaagaagaggccccagagggctacgtccaatgtcttcgccatgtttgaccagtcccagatccaggagtttaaggaggccttcaacatgattgatcagaaccgagatggcttcattgataaggaggacctgcacgacatgctggcctctctggggaagaaccccacagacgagtatctggagggcatgatgaacgaggcgccagggcccatcaacttcaccatgttcctcacaatgtttggggagaagctgaacggcacagaccccgaggatgtgatccgcaatgcctttgcctgctttgatgaggaggcctcaggcttcatccacgaggaccacctgagggagctgctcaccaccatgggcgaccgattcacggatgaggaggtggacgagatgtaccgcgaggcacccattgataagaagggcaacttcaactacgtggagttcactcgcatcctcaaacacggcgccaaggacaaggacgactaa

SEQ ID NO: 14 - protein, 172 aa, mus musculus
MSSKRAKAKTTKKRPQRATSNVFAMFDQSQIQEFKEAFNMIDQNRDGFIDKEDLHDMLASLGKNPTDEYLEGMMNEAPGPINFTMFLTMFGEKLNGTDPEDVIRNAFACFDEEASGFIHEDHLRELLTTMGDRFTDEEVDEMYREAPIDKKGNFNYVEFTRILKHGAKDKDD

SEQ ID NO: 15 - DNA, 519 bp, mus musculus
  misc_feature: nucleotide sequence of DNA encoding mouse myl12 isoform a
  CDS (1)..(519)
atgtctagcaaaagggcaaagaccaagaccaccaagaagcgccctcagcgcgcaacctccaatgtgttcgccatgtttgaccagtcccagatccaggagttcaaagaagcctttaacatgattgaccagaaccgggatggcttcattgacaaggaggacctgcacgacatgctggcgtcaatgggaaaaaacccaactgacgaatacctggacgccatgatgaacgaggccccgggccccatcaatttcaccatgttcctcaccatgtttggggagaagctgaacggcactgaccccgaggacgtcatcagaaacgccttcgcttgctttgatgaggaagccatcggcaccatccaggaggattacctgagggagctgctgaccaccatgggcgaccgcttcacagacgaggaggtggatgagctgtacagagaggcccccattgacaaaaaggggaacttcaactacattgagttcacacgcatcctgaagcacggcgcgaaagacaaagatgactga

SEQ ID NO: 16 - protein, 172 aa, mus musculus
MSSKRAKTKTTKKRPQRATSNVFAMFDQSQIQEFKEAFNMIDQNRDGFIDKEDLHDMLASMGKNPTDEYLDAMMNEAPGPINFTMFLTMFGEKLNGTDPEDVIRNAFACFDEEAIGTIQEDYLRELLTTMGDRFTDEEVDELYREAPIDKKGNFNYIEFTRILKHGAKDKDD

SEQ ID NO: 17 - DNA, 519 bp, mus musculus
  misc_feature: nucleotide sequence of DNA encoding mouse myl12 isoform b
  CDS (1)..(519)
atgtcgagcaaaaaagcgaagaccaagaccaccaagaagcgccctcagcgcgcaacctccaatgtgttcgccatgtttgaccagtcccagatccaggagttcaaagaggcctttaacatgattgaccagaaccgggatggcttcattgacaaggaggacctgcacgacatgctggcgtctctggggaagaatcccactgatgcctacctggacgccatgatgaacgaggccccgggccccatcaatttcaccatgttcctcaccatgtttggggagaagctaaacggcactgaccccgaggacgtcatcagaaacgccttcgcttgctttgatgaggaagccacaggcaccatccaggaggattacctgagggagctgctgaccaccatgggcgaccgcttcacagacgaggaagtggatgagctgtacagagaggcccccattgacaaaaaggggaacttcaactacattgagttcacacgcatcctgaagcacggcgcgaaagacaaagatgactga

SEQ ID NO: 18 - protein, 172 aa, mus musculus; identical to SEQ ID NO: 8

SEQ ID NO: 19 - DNA, 600 bp, homo sapiens
  misc_feature: nucleotide sequence of DNA encoding human CD69
  CDS (1)..(600)
atgagctctgaaaattgtttcgtagcagagaacagctctttgcatccggagagtggacaagaaaatgatgccaccagtccccatttctcaacacgtcatgaagggtccttccaagttcctgtcctgtgtgctgtaatgaatgtggtcttcatcaccattttaatcatagctctcattgccttatcagtgggccaatacaattgtccaggccaatacacattctcaatgccatcagacagccatgtttcttcatgctctgaggactgggttggctaccagaggaaatgctactttatttctactgtgaagaggagctggacttcagcccaaaatgcttgttctgaacatggtgctactcttgctgtcattgattctgaaaaggacatgaactttctaaaacgatacgcaggtagagaggaacactgggttggactgaaaaaggaacctggtcacccatggaagtggtcaaatggcaaagaatttaacaactggttcaacgttacagggtctgacaagtgtgtttttctgaaaaacacagaggtcagcagcatggaatgtgagaagaatttatactggatatgtaacaaaccttacaaataa

SEQ ID NO: 20 - protein, 199 aa, homo sapiens
MSSENCFVAENSSLHPESGQENDATSPHFSTRHEGSFQVPVLCAVMNVVFITILIIALIALSVGQYNCPGQYTFSMPSDSHVSSCSEDWVGYQRKCYFISTVKRSWTSAQNACSEHGATLAVIDSEKDMNFLKRYAGREEHWVGLKKEPGHPWKWSNGKEFNNWFNVTGSDKCVFLKNTEVSSMECEKNLYWICNKPYK

SEQ ID NO: 21 - protein, 8 aa, artificial
  tag peptide
DYKDDDDK

SEQ ID NO: 22 - DNA, 20 bp, artificial
  Designed oligonucleotide for use as a primer
ctaaggccaaccgtgaaaag

SEQ ID NO: 23 - DNA, 20 bp, artificial
  Designed oligonucleotide for use as a primer
accagaggcatacagggaca

SEQ ID NO: 24 - protein, 27 aa, Artificial
  an amino acid sequence highly homologous to a N-terminal partial amino acid sequence of Myl9, Myl12a, and Myl12 b
MSSKRAKAKTTKKRPQRATSNVFAMFD